European Patent Specification EP 3 743 526 B1, published March 12, 2025. Title: REAGENTS AND METHODS FOR BLOCKING NON-SPECIFIC INTERACTIONS WITH NUCLEIC ACIDS. Applicant: Tsai, Cheng-ting Robinson, Peter. The sequence listing filed with the application follows.

SEQUENCE LISTING (1 sequence)

SEQ ID NO: 1 - DNA, 50 bp, Artificial Sequence
  nucleic acid blocker
tcgtggaactatctagcggtgtacgtgagtgggcatgtagcaagagggtc